European Patent Specification EP 3 636 274 B1, published July 17, 2024. Title: COMPOSITIONS AND METHODS FOR MODULATING GAMMA-C-CYTOKINE ACTIVITY. Applicant: Tagaya, Yutaka Azimi, Nazli. The sequence listing filed with the application follows.

SEQUENCE LISTING (8 sequences)

SEQ ID NO: 1 - protein, 19 aa, Artificial Sequence
  BNZ-Gamma peptide
IKEFLQRFIHIVQSIINTS

SEQ ID NO: 2 - protein, 11 aa, Artificial Sequence
  Gamma-c-cytokine inhibitory peptide
  VARIANT (1)...(1): Xaa = Asp or Glu
  VARIANT (4)...(4): Xaa = Glu, Gln or Asn
  VARIANT (5)...(5): Xaa = Ser or Arg
  VARIANT (6)...(6): Xaa = any amino acid
  VARIANT (7)...(7): Xaa = Ile or Lys
  VARIANT (8)...(8): Xaa = any amino acid
  VARIANT (9)...(9): Xaa = Leu or Ile
  VARIANT (10)...(10): Xaa = any amino acid
XFLXXXXXXXQ

SEQ ID NO: 3 - protein, 19 aa, Artificial Sequence
  IL-15 D-helix peptide
IKEFLQSFVHIVQMFINTS

SEQ ID NO: 4 - protein, 20 aa, Artificial Sequence
  IL-2 D-helix peptide
IVEFLNRWITFCQSIISTLT

SEQ ID NO: 5 - protein, 21 aa, Artificial Sequence
  IL-21 D-helix peptide
PKEFLERFKSLLQKMIHQHLS

SEQ ID NO: 6 - protein, 21 aa, Artificial Sequence
  IL-4 D-helix peptide
LENFLERLKTIMREKYSKCSS

SEQ ID NO: 7 - protein, 21 aa, Artificial Sequence [sequence omitted]

SEQ ID NO: 8 - protein, 20 aa, Artificial Sequence
  IL-7 D-helix peptide
DLCFLKRLLQEIKTCWNKIL